European Patent Application EP 4 574 976 A1, published June 25, 2025. Title: NUCLEIC ACIDS FOR TRANSFECTION. Applicant: AGC Inc. Application JP. The sequence listing filed with the application follows.

SEQUENCE LISTING (2 sequences)

SEQ ID NO: 1 - DNA, 22 bp, synthetic construct
  source 1..22: mol_type = other DNA
agggttagggttagggttaggg

SEQ ID NO: 2 - DNA, 19 bp, synthetic construct
  source 1..19: mol_type = other DNA
tttttcagttgaccatata